European Patent Application EP 4 617 661 A1, published September 17, 2025. Title: A HIGH THROUGHPUT CELL-FREE EXPRESSION AND SCREENING MICROFLUIDIC PLATFORM FOR GPCR DRUG DISCOVERY. Applicant: ETH Zürich / ETH transfer. The sequence listing filed with the application follows.

SEQUENCE LISTING (3 sequences)

SEQ ID NO: 1 - protein, 729 aa, synthetic construct
MKTIIALSYIFCLVFAMAGVVHVSLAALLLLPMAPAMHSDCIFKKEQAMCLEKIQRANELMGFNDSSPGCPGMWDNITCWKPAHVGEMVLVSCAELFRIFNPDQVWETETIGESDFGDSNSLDLSDMGVVSRNCTEDGWSEPFPHYFDACGFDEYESETGDQDYYYLSVKALYTVGYSTSLVTLTTAMVILCRFRKLHCTRNFIHMNLFVSFMLRAISVFIKDWILYAEQDSNHCFISTVECKAVMVFFHYCVVSNYFWLFIEGLYLFTLLVETKKKERRYFYWYTIIGWGTPTVCVTVWATLRLYFDDTGCWDMNDSTALWWVIKGPVVGSIMVNFVLFIGIIVILVQKLQLSSLINVYIKADKQKNGIKANFKIRHNIEDGGVQLAYHYQQNTPIGDGPVLLPDNHYLSVQSKLSKDPNEKRDHMVLLEFVTAAGITLGMDELYKGGTGGSMVSKGEELFTGVVPILVELDGDVNGHKFSVSGEGEGDATYGKLTLKFICTTGKLPVPWPTLVTTLTYGVQCFSRYPDHMKQHDFFKSAMPEGYIQERTIFFKDDGNYKTRAEVKFEGDTLVNRIELKGIDFKEDGNILGHKLEYNNHDQLNESSIYLRLARSTLLLIPLFGIHYTVFAFSPENVSKRERLVFELGLGSFQGFVVAVLYCFLNGEVQAEIKRKWRSWKVNRYFAVDFKHRHPSLASSGVNGGTQLSILSKSSSQIRMSGLPADNLAA

SEQ ID NO: 2 - protein, 33 aa, Homo sp.
FTDSYSRYRKQMAVKKYLAAVLGKRYKQRVKNK

SEQ ID NO: 3 - protein, 38 aa, Homo sp.
HSDGIFTDSYSRYRKQMAVKKYLAAVLGKRYKQRVKNK